European Patent Application EP 4 745 162 A1, published May 20, 2026. Title: 一种表达融合蛋白的免疫细胞及其表达载体、应用和制备方法. Applicant: 乘典(苏州)生物医药有限公司. Application WO. The sequence listing filed with the application follows.

SEQUENCE LISTING (80 sequences)

SEQ ID NO: 1 - DNA, 1260 bp, synthetic construct
  source 1..1260: mol_type = other DNA
atgaccaggctgacagtgctggccctgctggcaggactgctggcaagctccagggccgaggtgcagctggtggagtccggcggcggcctggtgcagcctggagtatccctgaggctgtcttgcgcagcaagcggcttcacctttacatcctacaccatgtcttgggtgagacagaccccaggcaagggactggagtgggtggccttcatcagcggcggaggaggcgacacatactatcctgattccgtgaagggccggtttaccatcagcagagacaactccaagaatacactgtatctgcagatgaactccctgagggcagaggacaccgccgtgtactattgcgccagacacggctacgatggcacatggttcgcctattggggccagggcaccctggtgacagtgtctagcggaggaggaggatctggaggaggaggaagcggaggaggaggatccgacgtgctgacccagagcccatcctctctgtctgccagcgtgggcgatagggtgaccatcacatgtcgcgcctctgagaacatctacagctatctggcctggtaccagcagaagcccggcaagtcccctaagctgctggtgtctaatgcaaagaccctggcagagggagtgccatctaggttctccggctctggcagcggcacccagtttagcctgacaatcagctccctgcagcctgaggatttcgccacatactattgtcagcagcactacgccaccccatatacatttggcggcggcaccaagctggagatcaagaggacagtgggaggaggaggaagcggaggaggaggatccggcggcggcggctctcaaggtcaagatcgccacatgattagaatgcgtcaacttatagatattgttgatcagctgaaaaattatgtgaatgacttggtccctgaatttctgccagctccagaagatgtagagacaaactgtgagtggtcagctttttcctgttttcagaaggcccaactaaagtcagcaaatacaggaaacaatgaaaggataatcaatgtatctattaaaaagctgaagaggaacctctggggcctggcgggcttgaattcctgcccttcatgtgattcttatgagaaaaaaccacccaaagaattcctagaaagattcaaatcacttctccaaaagatgattcatcagcatctgtcctctagaacacacggaagtgaagattccgggggtggaggctctcaccatcaccaccatcatcaccaccatcactag

SEQ ID NO: 2 - protein, 419 aa, synthetic construct
MTRLTVLALLAGLLASSRAEVQLVESGGGLVQPGVSLRLSCAASGFTFTSYTMSWVRQTPGKGLEWVAFISGGGGDTYYPDSVKGRFTISRDNSKNTLYLQMNSLRAEDTAVYYCARHGYDGTWFAYWGQGTLVTVSSGGGGSGGGGSGGGGSDVLTQSPSSLSASVGDRVTITCRASENIYSYLAWYQQKPGKSPKLLVSNAKTLAEGVPSRFSGSGSGTQFSLTISSLQPEDFATYYCQQHYATPYTFGGGTKLEIKRTVGGGGSGGGGSGGGGSQGQDRHMIRMRQLIDIVDQLKNYVNDLVPEFLPAPEDVETNCEWSAFSCFQKAQLKSANTGNNERIINVSIKKLKRNLWGLAGLNSCPSCDSYEKKPPKEFLERFKSLLQKMIHQHLSSRTHGSEDSGGGGSHHHHHHHHHH

SEQ ID NO: 3 - DNA, 1215 bp, synthetic construct
  source 1..1215: mol_type = other DNA
atgaccaggctgacagtgctggccctgctggcaggactgctggcaagctccagggccgaggtgcagctggtggagtccggcggcggcctggtgcagcctggagtatccctgaggctgtcttgcgcagcaagcggcttcacctttacatcctacaccatgtcttgggtgagacagaccccaggcaagggactggagtgggtggccttcatcagcggcggaggaggcgacacatactatcctgattccgtgaagggccggtttaccatcagcagagacaactccaagaatacactgtatctgcagatgaactccctgagggcagaggacaccgccgtgtactattgcgccagacacggctacgatggcacatggttcgcctattggggccagggcaccctggtgacagtgtctagcggaggaggaggatctggaggaggaggaagcggaggaggaggatccgacgtgctgacccagagcccatcctctctgtctgccagcgtgggcgatagggtgaccatcacatgtcgcgcctctgagaacatctacagctatctggcctggtaccagcagaagcccggcaagtcccctaagctgctggtgtctaatgcaaagaccctggcagagggagtgccatctaggttctccggctctggcagcggcacccagtttagcctgacaatcagctccctgcagcctgaggatttcgccacatactattgtcagcagcactacgccaccccatatacatttggcggcggcaccaagctggagatcaagaggacagtgggaggaggaggaagcggaggaggaggatccggcggcggcggctctcaaggtcaagatcgccacatgattagaatgcgtcaacttatagatattgttgatcagctgaaaaattatgtgaatgacttggtccctgaatttctgccagctccagaagatgtagagacaaactgtgagtggtcagctttttcctgttttcagaaggcccaactaaagtcagcaaatacaggaaacaatgaaaggataatcaatgtatctattaaaaagctgaagaggaacctctggggcctggcgggcttgaattcctgcccttcatgtgattcttatgagaaaaaaccacccaaagaattcctagaaagattcaaatcacttctccaaaagatgattcatcagcatctgtcctctagaacacacggaagtgaagattccggg

SEQ ID NO: 4 - protein, 404 aa, synthetic construct
MTRLTVLALLAGLLASSRAEVQLVESGGGLVQPGVSLRLSCAASGFTFTSYTMSWVRQTPGKGLEWVAFISGGGGDTYYPDSVKGRFTISRDNSKNTLYLQMNSLRAEDTAVYYCARHGYDGTWFAYWGQGTLVTVSSGGGGSGGGGSGGGGSDVLTQSPSSLSASVGDRVTITCRASENIYSYLAWYQQKPGKSPKLLVSNAKTLAEGVPSRFSGSGSGTQFSLTISSLQPEDFATYYCQQHYATPYTFGGGTKLEIKRTVGGGGSGGGGSGGGGSQGQDRHMIRMRQLIDIVDQLKNYVNDLVPEFLPAPEDVETNCEWSAFSCFQKAQLKSANTGNNERIINVSIKKLKRNLWGLAGLNSCPSCDSYEKKPPKEFLERFKSLLQKMIHQHLSSRTHGSEDS

SEQ ID NO: 5 - DNA, 786 bp, synthetic construct
  source 1..786: mol_type = other DNA
atgaccaggctgacagtgctggccctgctggcaggactgctggcaagctccagggccgaggtgcagctggtggagtccggcggcggcctggtgcagcctggagtatccctgaggctgtcttgcgcagcaagcggcttcacctttacatcctacaccatgtcttgggtgagacagaccccaggcaagggactggagtgggtggccttcatcagcggcggaggaggcgacacatactatcctgattccgtgaagggccggtttaccatcagcagagacaactccaagaatacactgtatctgcagatgaactccctgagggcagaggacaccgccgtgtactattgcgccagacacggctacgatggcacatggttcgcctattggggccagggcaccctggtgacagtgtctagcggaggaggaggatctggaggaggaggaagcggaggaggaggatccgacgtgctgacccagagcccatcctctctgtctgccagcgtgggcgatagggtgaccatcacatgtcgcgcctctgagaacatctacagctatctggcctggtaccagcagaagcccggcaagtcccctaagctgctggtgtctaatgcaaagaccctggcagagggagtgccatctaggttctccggctctggcagcggcacccagtttagcctgacaatcagctccctgcagcctgaggatttcgccacatactattgtcagcagcactacgccaccccatatacatttggcggcggcaccaagctggagatcaagaggacagtg

SEQ ID NO: 6 - protein, 262 aa, synthetic construct
MTRLTVLALLAGLLASSRAEVQLVESGGGLVQPGVSLRLSCAASGFTFTSYTMSWVRQTPGKGLEWVAFISGGGGDTYYPDSVKGRFTISRDNSKNTLYLQMNSLRAEDTAVYYCARHGYDGTWFAYWGQGTLVTVSSGGGGSGGGGSGGGGSDVLTQSPSSLSASVGDRVTITCRASENIYSYLAWYQQKPGKSPKLLVSNAKTLAEGVPSRFSGSGSGTQFSLTISSLQPEDFATYYCQQHYATPYTFGGGTKLEIKRTV

SEQ ID NO: 7 - DNA, 414 bp, synthetic construct
  source 1..414: mol_type = other DNA
atgaccaggctgacagtgctggccctgctggcaggactgctggcaagctccagggccgaggtgcagctggtggagtccggcggcggcctggtgcagcctggagtatccctgaggctgtcttgcgcagcaagcggcttcacctttacatcctacaccatgtcttgggtgagacagaccccaggcaagggactggagtgggtggccttcatcagcggcggaggaggcgacacatactatcctgattccgtgaagggccggtttaccatcagcagagacaactccaagaatacactgtatctgcagatgaactccctgagggcagaggacaccgccgtgtactattgcgccagacacggctacgatggcacatggttcgcctattggggccagggcaccctggtgacagtgtctagc

SEQ ID NO: 8 - protein, 138 aa, synthetic construct
MTRLTVLALLAGLLASSRAEVQLVESGGGLVQPGVSLRLSCAASGFTFTSYTMSWVRQTPGKGLEWVAFISGGGGDTYYPDSVKGRFTISRDNSKNTLYLQMNSLRAEDTAVYYCARHGYDGTWFAYWGQGTLVTVSS

SEQ ID NO: 9 - DNA, 45 bp, synthetic construct
  source 1..45: mol_type = other DNA
ggaggaggaggatctggaggaggaggaagcggaggaggaggatcc

SEQ ID NO: 10 - protein, 15 aa, synthetic construct
GGGGSGGGGSGGGGS

SEQ ID NO: 11 - DNA, 327 bp, synthetic construct
  source 1..327: mol_type = other DNA
gacgtgctgacccagagcccatcctctctgtctgccagcgtgggcgatagggtgaccatcacatgtcgcgcctctgagaacatctacagctatctggcctggtaccagcagaagcccggcaagtcccctaagctgctggtgtctaatgcaaagaccctggcagagggagtgccatctaggttctccggctctggcagcggcacccagtttagcctgacaatcagctccctgcagcctgaggatttcgccacatactattgtcagcagcactacgccaccccatatacatttggcggcggcaccaagctggagatcaagaggacagtg

SEQ ID NO: 12 - protein, 109 aa, synthetic construct
DVLTQSPSSLSASVGDRVTITCRASENIYSYLAWYQQKPGKSPKLLVSNAKTLAEGVPSRFSGSGSGTQFSLTISSLQPEDFATYYCQQHYATPYTFGGGTKLEIKRTV

SEQ ID NO: 13 - DNA, 45 bp, synthetic construct
  source 1..45: mol_type = other DNA
ggaggaggaggaagcggaggaggaggatccggcggcggcggctct

SEQ ID NO: 14 - protein, 15 aa, synthetic construct
GGGGSGGGGSGGGGS

SEQ ID NO: 15 - DNA, 381 bp, Homo sapiens
  source 1..381: mol_type = other DNA
caaggtcaagatcgccacatgattagaatgcgtcaacttatagatattgttgatcagctgaaaaattatgtgaatgacttggtccctgaatttctgccagctccagaagatgtagagacaaactgtgagtggtcagctttttcctgttttcagaaggcccaactaaagtcagcaaatacaggaaacaatgaaaggataatcaatgtatctattaaaaagctgaagaggaacctctggggcctggcgggcttgaattcctgcccttcatgtgattcttatgagaaaaaaccacccaaagaattcctagaaagattcaaatcacttctccaaaagatgattcatcagcatctgtcctctagaacacacggaagtgaagattcc

SEQ ID NO: 16 - protein, 127 aa, Homo sapiens
QGQDRHMIRMRQLIDIVDQLKNYVNDLVPEFLPAPEDVETNCEWSAFSCFQKAQLKSANTGNNERIINVSIKKLKRNLWGLAGLNSCPSCDSYEKKPPKEFLERFKSLLQKMIHQHLSSRTHGSEDS

SEQ ID NO: 17 - DNA, 15 bp, synthetic construct
  source 1..15: mol_type = other DNA
gggggtggaggctct

SEQ ID NO: 18 - protein, 5 aa, synthetic construct
GGGGS

SEQ ID NO: 19 - DNA, 2844 bp, synthetic construct
  source 1..2844: mol_type = other DNA
atgcttctcctggtgacaagccttctgctctgtgagttaccacacccagcattcctcctgatcccagacatccagatgacacagactacatcctccctgtctgcctctctgggagacagagtcaccatcagttgcagggcaagtcaggacattagtaaatatttaaattggtatcagcagaaaccagatggaactgttaaactcctgatctaccatacatcaagattacactcaggagtcccatcaaggttcagtggcagtgggtctggaacagattattctctcaccattagcaacctggagcaagaagatattgccacttacttttgccaacagggtaatacgcttccgtacacgttcggaggggggactaagttggaaataacaggctccacctctggatccggcaagcccggatctggcgagggatccaccaagggcgaggtgaaactgcaggagtcaggacctggcctggtggcgccctcacagagcctgtccgtcacatgcactgtctcaggggtctcattacccgactatggtgtaagctggattcgccagcctccacgaaagggtctggagtggctgggagtaatatggggtagtgaaaccacatactataattcagctctcaaatccagactgaccatcatcaaggacaactccaagagccaagttttcttaaaaatgaacagtctgcaaactgatgacacagccatttactactgtgccaaacattattactacggtggtagctatgctatggactactggggtcaaggaacctcagtcaccgtctcctcagcggccgcattcgtgccggtcttcctgccagcgaagcccaccacgacgccagcgccgcgaccaccaacaccggcgcccaccatcgcgtcgcagcccctgtccctgcgcccagaggcgtgccggccagcggcggggggcgcagtgcacacgagggggctggacttcgcctgtgatatctacatctgggcgcccttggccgggacttgtggggtccttctcctgtcactggttatcaccctttactgcaaccacaggaacaaacggggcagaaagaaactcctgtatatattcaaacaaccatttatgagaccagtacaaactactcaagaggaagatggctgtagctgccgatttccagaagaagaagaaggaggatgtgaactgagagtgaagttcagcaggagcgcagagccccccgcgtaccagcagggccagaaccagctctataacgagctcaatctaggacgaagagaggagtacgatgttttggacaagagacgtggccgggaccctgagatggggggaaagccgagaaggaagaaccctcaggaaggcctgtacaatgaactgcagaaagataagatggcggaggcctacagtgagattgggatgaaaggcgagcgccggaggggcaaggggcacgatggcctttaccagggtctcagtacagccaccaaggacacctacgacgcccttcacatgcaggccctgccccctcgcggcagtggagagggcagaggaagtctgctaacatgcggtgacgtcgaggagaatcctggcccaatgaccaggctgacagtgctggccctgctggcaggactgctggcaagctccagggccgaggtgcagctggtggagtccggcggcggcctggtgcagcctggagtatccctgaggctgtcttgcgcagcaagcggcttcacctttacatcctacaccatgtcttgggtgagacagaccccaggcaagggactggagtgggtggccttcatcagcggcggaggaggcgacacatactatcctgattccgtgaagggccggtttaccatcagcagagacaactccaagaatacactgtatctgcagatgaactccctgagggcagaggacaccgccgtgtactattgcgccagacacggctacgatggcacatggttcgcctattggggccagggcaccctggtgacagtgtctagcggaggaggaggatctggaggaggaggaagcggaggaggaggatccgacgtgctgacccagagcccatcctctctgtctgccagcgtgggcgatagggtgaccatcacatgtcgcgcctctgagaacatctacagctatctggcctggtaccagcagaagcccggcaagtcccctaagctgctggtgtctaatgcaaagaccctggcagagggagtgccatctaggttctccggctctggcagcggcacccagtttagcctgacaatcagctccctgcagcctgaggatttcgccacatactattgtcagcagcactacgccaccccatatacatttggcggcggcaccaagctggagatcaagaggacagtgggaggaggaggaagcggaggaggaggatccggcggcggcggctctcaaggtcaagatcgccacatgattagaatgcgtcaacttatagatattgttgatcagctgaaaaattatgtgaatgacttggtccctgaatttctgccagctccagaagatgtagagacaaactgtgagtggtcagctttttcctgttttcagaaggcccaactaaagtcagcaaatacaggaaacaatgaaaggataatcaatgtatctattaaaaagctgaagaggaacctctggggcctggcgggcttgaattcctgcccttcatgtgattcttatgagaaaaaaccacccaaagaattcctagaaagattcaaatcacttctccaaaagatgattcatcagcatctgtcctctagaacacacggaagtgaagattccgggggtggaggctctcaccatcaccaccatcatcaccaccatcactag

SEQ ID NO: 20 - protein, 947 aa, synthetic construct
MLLLVTSLLLCELPHPAFLLIPDIQMTQTTSSLSASLGDRVTISCRASQDISKYLNWYQQKPDGTVKLLIYHTSRLHSGVPSRFSGSGSGTDYSLTISNLEQEDIATYFCQQGNTLPYTFGGGTKLEITGSTSGSGKPGSGEGSTKGEVKLQESGPGLVAPSQSLSVTCTVSGVSLPDYGVSWIRQPPRKGLEWLGVIWGSETTYYNSALKSRLTIIKDNSKSQVFLKMNSLQTDDTAIYYCAKHYYYGGSYAMDYWGQGTSVTVSSAAAFVPVFLPAKPTTTPAPRPPTPAPTIASQPLSLRPEACRPAAGGAVHTRGLDFACDIYIWAPLAGTCGVLLLSLVITLYCNHRNKRGRKKLLYIFKQPFMRPVQTTQEEDGCSCRFPEEEEGGCELRVKFSRSAEPPAYQQGQNQLYNELNLGRREEYDVLDKRRGRDPEMGGKPRRKNPQEGLYNELQKDKMAEAYSEIGMKGERRRGKGHDGLYQGLSTATKDTYDALHMQALPPRGSGEGRGSLLTCGDVEENPGPMTRLTVLALLAGLLASSRAEVQLVESGGGLVQPGVSLRLSCAASGFTFTSYTMSWVRQTPGKGLEWVAFISGGGGDTYYPDSVKGRFTISRDNSKNTLYLQMNSLRAEDTAVYYCARHGYDGTWFAYWGQGTLVTVSSGGGGSGGGGSGGGGSDVLTQSPSSLSASVGDRVTITCRASENIYSYLAWYQQKPGKSPKLLVSNAKTLAEGVPSRFSGSGSGTQFSLTISSLQPEDFATYYCQQHYATPYTFGGGTKLEIKRTVGGGGSGGGGSGGGGSQGQDRHMIRMRQLIDIVDQLKNYVNDLVPEFLPAPEDVETNCEWSAFSCFQKAQLKSANTGNNERIINVSIKKLKRNLWGLAGLNSCPSCDSYEKKPPKEFLERFKSLLQKMIHQHLSSRTHGSEDSGGGGSHHHHHHHHHH

SEQ ID NO: 21 - DNA, 2799 bp, synthetic construct
  source 1..2799: mol_type = other DNA
atgcttctcctggtgacaagccttctgctctgtgagttaccacacccagcattcctcctgatcccagacatccagatgacacagactacatcctccctgtctgcctctctgggagacagagtcaccatcagttgcagggcaagtcaggacattagtaaatatttaaattggtatcagcagaaaccagatggaactgttaaactcctgatctaccatacatcaagattacactcaggagtcccatcaaggttcagtggcagtgggtctggaacagattattctctcaccattagcaacctggagcaagaagatattgccacttacttttgccaacagggtaatacgcttccgtacacgttcggaggggggactaagttggaaataacaggctccacctctggatccggcaagcccggatctggcgagggatccaccaagggcgaggtgaaactgcaggagtcaggacctggcctggtggcgccctcacagagcctgtccgtcacatgcactgtctcaggggtctcattacccgactatggtgtaagctggattcgccagcctccacgaaagggtctggagtggctgggagtaatatggggtagtgaaaccacatactataattcagctctcaaatccagactgaccatcatcaaggacaactccaagagccaagttttcttaaaaatgaacagtctgcaaactgatgacacagccatttactactgtgccaaacattattactacggtggtagctatgctatggactactggggtcaaggaacctcagtcaccgtctcctcagcggccgcattcgtgccggtcttcctgccagcgaagcccaccacgacgccagcgccgcgaccaccaacaccggcgcccaccatcgcgtcgcagcccctgtccctgcgcccagaggcgtgccggccagcggcggggggcgcagtgcacacgagggggctggacttcgcctgtgatatctacatctgggcgcccttggccgggacttgtggggtccttctcctgtcactggttatcaccctttactgcaaccacaggaacaaacggggcagaaagaaactcctgtatatattcaaacaaccatttatgagaccagtacaaactactcaagaggaagatggctgtagctgccgatttccagaagaagaagaaggaggatgtgaactgagagtgaagttcagcaggagcgcagagccccccgcgtaccagcagggccagaaccagctctataacgagctcaatctaggacgaagagaggagtacgatgttttggacaagagacgtggccgggaccctgagatggggggaaagccgagaaggaagaaccctcaggaaggcctgtacaatgaactgcagaaagataagatggcggaggcctacagtgagattgggatgaaaggcgagcgccggaggggcaaggggcacgatggcctttaccagggtctcagtacagccaccaaggacacctacgacgcccttcacatgcaggccctgccccctcgcggcagtggagagggcagaggaagtctgctaacatgcggtgacgtcgaggagaatcctggcccaatgaccaggctgacagtgctggccctgctggcaggactgctggcaagctccagggccgaggtgcagctggtggagtccggcggcggcctggtgcagcctggagtatccctgaggctgtcttgcgcagcaagcggcttcacctttacatcctacaccatgtcttgggtgagacagaccccaggcaagggactggagtgggtggccttcatcagcggcggaggaggcgacacatactatcctgattccgtgaagggccggtttaccatcagcagagacaactccaagaatacactgtatctgcagatgaactccctgagggcagaggacaccgccgtgtactattgcgccagacacggctacgatggcacatggttcgcctattggggccagggcaccctggtgacagtgtctagcggaggaggaggatctggaggaggaggaagcggaggaggaggatccgacgtgctgacccagagcccatcctctctgtctgccagcgtgggcgatagggtgaccatcacatgtcgcgcctctgagaacatctacagctatctggcctggtaccagcagaagcccggcaagtcccctaagctgctggtgtctaatgcaaagaccctggcagagggagtgccatctaggttctccggctctggcagcggcacccagtttagcctgacaatcagctccctgcagcctgaggatttcgccacatactattgtcagcagcactacgccaccccatatacatttggcggcggcaccaagctggagatcaagaggacagtgggaggaggaggaagcggaggaggaggatccggcggcggcggctctcaaggtcaagatcgccacatgattagaatgcgtcaacttatagatattgttgatcagctgaaaaattatgtgaatgacttggtccctgaatttctgccagctccagaagatgtagagacaaactgtgagtggtcagctttttcctgttttcagaaggcccaactaaagtcagcaaatacaggaaacaatgaaaggataatcaatgtatctattaaaaagctgaagaggaacctctggggcctggcgggcttgaattcctgcccttcatgtgattcttatgagaaaaaaccacccaaagaattcctagaaagattcaaatcacttctccaaaagatgattcatcagcatctgtcctctagaacacacggaagtgaagattcctag

SEQ ID NO: 22 - protein, 932 aa, synthetic construct
MLLLVTSLLLCELPHPAFLLIPDIQMTQTTSSLSASLGDRVTISCRASQDISKYLNWYQQKPDGTVKLLIYHTSRLHSGVPSRFSGSGSGTDYSLTISNLEQEDIATYFCQQGNTLPYTFGGGTKLEITGSTSGSGKPGSGEGSTKGEVKLQESGPGLVAPSQSLSVTCTVSGVSLPDYGVSWIRQPPRKGLEWLGVIWGSETTYYNSALKSRLTIIKDNSKSQVFLKMNSLQTDDTAIYYCAKHYYYGGSYAMDYWGQGTSVTVSSAAAFVPVFLPAKPTTTPAPRPPTPAPTIASQPLSLRPEACRPAAGGAVHTRGLDFACDIYIWAPLAGTCGVLLLSLVITLYCNHRNKRGRKKLLYIFKQPFMRPVQTTQEEDGCSCRFPEEEEGGCELRVKFSRSAEPPAYQQGQNQLYNELNLGRREEYDVLDKRRGRDPEMGGKPRRKNPQEGLYNELQKDKMAEAYSEIGMKGERRRGKGHDGLYQGLSTATKDTYDALHMQALPPRGSGEGRGSLLTCGDVEENPGPMTRLTVLALLAGLLASSRAEVQLVESGGGLVQPGVSLRLSCAASGFTFTSYTMSWVRQTPGKGLEWVAFISGGGGDTYYPDSVKGRFTISRDNSKNTLYLQMNSLRAEDTAVYYCARHGYDGTWFAYWGQGTLVTVSSGGGGSGGGGSGGGGSDVLTQSPSSLSASVGDRVTITCRASENIYSYLAWYQQKPGKSPKLLVSNAKTLAEGVPSRFSGSGSGTQFSLTISSLQPEDFATYYCQQHYATPYTFGGGTKLEIKRTVGGGGSGGGGSGGGGSQGQDRHMIRMRQLIDIVDQLKNYVNDLVPEFLPAPEDVETNCEWSAFSCFQKAQLKSANTGNNERIINVSIKKLKRNLWGLAGLNSCPSCDSYEKKPPKEFLERFKSLLQKMIHQHLSSRTHGSEDS

SEQ ID NO: 23 - DNA, 66 bp, synthetic construct
  source 1..66: mol_type = other DNA
atgcttctcctggtgacaagccttctgctctgtgagttaccacacccagcattcctcctgatccca

SEQ ID NO: 24 - protein, 22 aa, synthetic construct
MLLLVTSLLLCELPHPAFLLIP

SEQ ID NO: 25 - DNA, 321 bp, synthetic construct
  source 1..321: mol_type = other DNA
gacatccagatgacacagactacatcctccctgtctgcctctctgggagacagagtcaccatcagttgcagggcaagtcaggacattagtaaatatttaaattggtatcagcagaaaccagatggaactgttaaactcctgatctaccatacatcaagattacactcaggagtcccatcaaggttcagtggcagtgggtctggaacagattattctctcaccattagcaacctggagcaagaagatattgccacttacttttgccaacagggtaatacgcttccgtacacgttcggaggggggactaagttggaaataaca

SEQ ID NO: 26 - protein, 107 aa, synthetic construct
DIQMTQTTSSLSASLGDRVTISCRASQDISKYLNWYQQKPDGTVKLLIYHTSRLHSGVPSRFSGSGSGTDYSLTISNLEQEDIATYFCQQGNTLPYTFGGGTKLEIT

SEQ ID NO: 27 - DNA, 54 bp, synthetic construct
  source 1..54: mol_type = other DNA
ggctccacctctggatccggcaagcccggatctggcgagggatccaccaagggc

SEQ ID NO: 28 - protein, 18 aa, synthetic construct
GSTSGSGKPGSGEGSTKG

SEQ ID NO: 29 - DNA, 360 bp, synthetic construct
  source 1..360: mol_type = other DNA
gaggtgaaactgcaggagtcaggacctggcctggtggcgccctcacagagcctgtccgtcacatgcactgtctcaggggtctcattacccgactatggtgtaagctggattcgccagcctccacgaaagggtctggagtggctgggagtaatatggggtagtgaaaccacatactataattcagctctcaaatccagactgaccatcatcaaggacaactccaagagccaagttttcttaaaaatgaacagtctgcaaactgatgacacagccatttactactgtgccaaacattattactacggtggtagctatgctatggactactggggtcaaggaacctcagtcaccgtctcctca

SEQ ID NO: 30 - protein, 120 aa, synthetic construct
EVKLQESGPGLVAPSQSLSVTCTVSGVSLPDYGVSWIRQPPRKGLEWLGVIWGSETTYYNSALKSRLTIIKDNSKSQVFLKMNSLQTDDTAIYYCAKHYYYGGSYAMDYWGQGTSVTVSS

SEQ ID NO: 31 - DNA, 735 bp, synthetic construct
  source 1..735: mol_type = other DNA
gacatccagatgacacagactacatcctccctgtctgcctctctgggagacagagtcaccatcagttgcagggcaagtcaggacattagtaaatatttaaattggtatcagcagaaaccagatggaactgttaaactcctgatctaccatacatcaagattacactcaggagtcccatcaaggttcagtggcagtgggtctggaacagattattctctcaccattagcaacctggagcaagaagatattgccacttacttttgccaacagggtaatacgcttccgtacacgttcggaggggggactaagttggaaataacaggctccacctctggatccggcaagcccggatctggcgagggatccaccaagggcgaggtgaaactgcaggagtcaggacctggcctggtggcgccctcacagagcctgtccgtcacatgcactgtctcaggggtctcattacccgactatggtgtaagctggattcgccagcctccacgaaagggtctggagtggctgggagtaatatggggtagtgaaaccacatactataattcagctctcaaatccagactgaccatcatcaaggacaactccaagagccaagttttcttaaaaatgaacagtctgcaaactgatgacacagccatttactactgtgccaaacattattactacggtggtagctatgctatggactactggggtcaaggaacctcagtcaccgtctcctca

SEQ ID NO: 32 - protein, 245 aa, synthetic construct
DIQMTQTTSSLSASLGDRVTISCRASQDISKYLNWYQQKPDGTVKLLIYHTSRLHSGVPSRFSGSGSGTDYSLTISNLEQEDIATYFCQQGNTLPYTFGGGTKLEITGSTSGSGKPGSGEGSTKGEVKLQESGPGLVAPSQSLSVTCTVSGVSLPDYGVSWIRQPPRKGLEWLGVIWGSETTYYNSALKSRLTIIKDNSKSQVFLKMNSLQTDDTAIYYCAKHYYYGGSYAMDYWGQGTSVTVSS

SEQ ID NO: 33 - DNA, 174 bp, synthetic construct
  source 1..174: mol_type = other DNA
gcggccgcattcgtgccggtcttcctgccagcgaagcccaccacgacgccagcgccgcgaccaccaacaccggcgcccaccatcgcgtcgcagcccctgtccctgcgcccagaggcgtgccggccagcggcggggggcgcagtgcacacgagggggctggacttcgcctgtgat

SEQ ID NO: 34 - protein, 58 aa, synthetic construct
AAAFVPVFLPAKPTTTPAPRPPTPAPTIASQPLSLRPEACRPAAGGAVHTRGLDFACD

SEQ ID NO: 35 - DNA, 84 bp, synthetic construct
  source 1..84: mol_type = other DNA
atctacatctgggcgcccttggccgggacttgtggggtccttctcctgtcactggttatcaccctttactgcaaccacaggaac

SEQ ID NO: 36 - protein, 28 aa, synthetic construct
IYIWAPLAGTCGVLLLSLVITLYCNHRN

SEQ ID NO: 37 - DNA, 126 bp, synthetic construct
  source 1..126: mol_type = other DNA
aaacggggcagaaagaaactcctgtatatattcaaacaaccatttatgagaccagtacaaactactcaagaggaagatggctgtagctgccgatttccagaagaagaagaaggaggatgtgaactg

SEQ ID NO: 38 - protein, 42 aa, synthetic construct
KRGRKKLLYIFKQPFMRPVQTTQEEDGCSCRFPEEEEGGCEL

SEQ ID NO: 39 - DNA, 336 bp, synthetic construct
  source 1..336: mol_type = other DNA
agagtgaagttcagcaggagcgcagagccccccgcgtaccagcagggccagaaccagctctataacgagctcaatctaggacgaagagaggagtacgatgttttggacaagagacgtggccgggaccctgagatggggggaaagccgagaaggaagaaccctcaggaaggcctgtacaatgaactgcagaaagataagatggcggaggcctacagtgagattgggatgaaaggcgagcgccggaggggcaaggggcacgatggcctttaccagggtctcagtacagccaccaaggacacctacgacgcccttcacatgcaggccctgccccctcgc

SEQ ID NO: 40 - protein, 112 aa, synthetic construct
RVKFSRSAEPPAYQQGQNQLYNELNLGRREEYDVLDKRRGRDPEMGGKPRRKNPQEGLYNELQKDKMAEAYSEIGMKGERRRGKGHDGLYQGLSTATKDTYDALHMQALPPR

SEQ ID NO: 41 - DNA, 63 bp, synthetic construct
  source 1..63: mol_type = other DNA
ggcagtggagagggcagaggaagtctgctaacatgcggtgacgtcgaggagaatcctggccca

SEQ ID NO: 42 - protein, 21 aa, synthetic construct
GSGEGRGSLLTCGDVEENPGP

SEQ ID NO: 43 - DNA, 1524 bp, synthetic construct
  source 1..1524: mol_type = other DNA
atgcttctcctggtgacaagccttctgctctgtgagttaccacacccagcattcctcctgatcccagacatccagatgacacagactacatcctccctgtctgcctctctgggagacagagtcaccatcagttgcagggcaagtcaggacattagtaaatatttaaattggtatcagcagaaaccagatggaactgttaaactcctgatctaccatacatcaagattacactcaggagtcccatcaaggttcagtggcagtgggtctggaacagattattctctcaccattagcaacctggagcaagaagatattgccacttacttttgccaacagggtaatacgcttccgtacacgttcggaggggggactaagttggaaataacaggctccacctctggatccggcaagcccggatctggcgagggatccaccaagggcgaggtgaaactgcaggagtcaggacctggcctggtggcgccctcacagagcctgtccgtcacatgcactgtctcaggggtctcattacccgactatggtgtaagctggattcgccagcctccacgaaagggtctggagtggctgggagtaatatggggtagtgaaaccacatactataattcagctctcaaatccagactgaccatcatcaaggacaactccaagagccaagttttcttaaaaatgaacagtctgcaaactgatgacacagccatttactactgtgccaaacattattactacggtggtagctatgctatggactactggggtcaaggaacctcagtcaccgtctcctcagcggccgcattcgtgccggtcttcctgccagcgaagcccaccacgacgccagcgccgcgaccaccaacaccggcgcccaccatcgcgtcgcagcccctgtccctgcgcccagaggcgtgccggccagcggcggggggcgcagtgcacacgagggggctggacttcgcctgtgatatctacatctgggcgcccttggccgggacttgtggggtccttctcctgtcactggttatcaccctttactgcaaccacaggaacaaacggggcagaaagaaactcctgtatatattcaaacaaccatttatgagaccagtacaaactactcaagaggaagatggctgtagctgccgatttccagaagaagaagaaggaggatgtgaactgagagtgaagttcagcaggagcgcagagccccccgcgtaccagcagggccagaaccagctctataacgagctcaatctaggacgaagagaggagtacgatgttttggacaagagacgtggccgggaccctgagatggggggaaagccgagaaggaagaaccctcaggaaggcctgtacaatgaactgcagaaagataagatggcggaggcctacagtgagattgggatgaaaggcgagcgccggaggggcaaggggcacgatggcctttaccagggtctcagtacagccaccaaggacacctacgacgcccttcacatgcaggccctgccccctcgctaa

SEQ ID NO: 44 - protein, 507 aa, synthetic construct
MLLLVTSLLLCELPHPAFLLIPDIQMTQTTSSLSASLGDRVTISCRASQDISKYLNWYQQKPDGTVKLLIYHTSRLHSGVPSRFSGSGSGTDYSLTISNLEQEDIATYFCQQGNTLPYTFGGGTKLEITGSTSGSGKPGSGEGSTKGEVKLQESGPGLVAPSQSLSVTCTVSGVSLPDYGVSWIRQPPRKGLEWLGVIWGSETTYYNSALKSRLTIIKDNSKSQVFLKMNSLQTDDTAIYYCAKHYYYGGSYAMDYWGQGTSVTVSSAAAFVPVFLPAKPTTTPAPRPPTPAPTIASQPLSLRPEACRPAAGGAVHTRGLDFACDIYIWAPLAGTCGVLLLSLVITLYCNHRNKRGRKKLLYIFKQPFMRPVQTTQEEDGCSCRFPEEEEGGCELRVKFSRSAEPPAYQQGQNQLYNELNLGRREEYDVLDKRRGRDPEMGGKPRRKNPQEGLYNELQKDKMAEAYSEIGMKGERRRGKGHDGLYQGLSTATKDTYDALHMQALPPR

SEQ ID NO: 45 - DNA, 735 bp, synthetic construct
  source 1..735: mol_type = other DNA
attgtgctcactcagtcacctcccagcctggccatgagcctgggaaaaagggccaccatctcctgtagagccagtgagtccgtcacaatcttggggagccatcttattcactggtatcagcagaagcccgggcagcctccaacccttcttattcagctcgcgtcaaacgtccagacgggtgtacctgccagattttctggtagcgggtcccgcactgattttacactgaccatagatccagtggaagaagacgatgtggccgtgtattattgtctgcagagcagaacgattcctcgcacatttggtgggggtactaagctggagattaagggaagcacgtccggctcagggaagccgggctccggcgagggaagcacgaaggggcaaattcagctggtccagagcggacctgagctgaaaaaacccggcgagactgttaagatcagttgtaaagcatctggctataccttcaccgactacagcataaattgggtgaaacgggcccctggaaagggcctcaaatggatgggttggatcaataccgaaactagggagcctgcttatgcatatgacttccgcgggagattcgccttttcactcgagacatctgcctctactgcttacctccaaataaacaacctcaagtatgaagatacagccacttacttttgcgccctcgactatagttacgccatggactactggggacagggaacctccgttaccgtcagttcc

SEQ ID NO: 46 - protein, 245 aa, synthetic construct
IVLTQSPPSLAMSLGKRATISCRASESVTILGSHLIHWYQQKPGQPPTLLIQLASNVQTGVPARFSGSGSRTDFTLTIDPVEEDDVAVYYCLQSRTIPRTFGGGTKLEIKGSTSGSGKPGSGEGSTKGQIQLVQSGPELKKPGETVKISCKASGYTFTDYSINWVKRAPGKGLKWMGWINTETREPAYAYDFRGRFAFSLETSASTAYLQINNLKYEDTATYFCALDYSYAMDYWGQGTSVTVSS

SEQ ID NO: 47 - DNA, 330 bp, synthetic construct
  source 1..330: mol_type = other DNA
attgtgctcactcagtcacctcccagcctggccatgagcctgggaaaaagggccaccatctcctgtagagccagtgagtccgtcacaatcttggggagccatcttattcactggtatcagcagaagcccgggcagcctccaacccttcttattcagctcgcgtcaaacgtccagacgggtgtacctgccagattttctggtagcgggtcccgcactgattttacactgaccatagatccagtggaagaagacgatgtggccgtgtattattgtctgcagagcagaacgattcctcgcacatttggtgggggtactaagctggagattaag

SEQ ID NO: 48 - protein, 110 aa, synthetic construct
IVLTQSPPSLAMSLGKRATISCRASESVTILGSHLIHWYQQKPGQPPTLLIQLASNVQTGVPARFSGSGSRTDFTLTIDPVEEDDVAVYYCLQSRTIPRTFGGGTKLEIK

SEQ ID NO: 49 - DNA, 54 bp, synthetic construct
  source 1..54: mol_type = other DNA
ggaagcacgtccggctcagggaagccgggctccggcgagggaagcacgaagggg

SEQ ID NO: 50 - protein, 18 aa, synthetic construct
GSTSGSGKPGSGEGSTKG

SEQ ID NO: 51 - DNA, 351 bp, synthetic construct
  source 1..351: mol_type = other DNA
caaattcagctggtccagagcggacctgagctgaaaaaacccggcgagactgttaagatcagttgtaaagcatctggctataccttcaccgactacagcataaattgggtgaaacgggcccctggaaagggcctcaaatggatgggttggatcaataccgaaactagggagcctgcttatgcatatgacttccgcgggagattcgccttttcactcgagacatctgcctctactgcttacctccaaataaacaacctcaagtatgaagatacagccacttacttttgcgccctcgactatagttacgccatggactactggggacagggaacctccgttaccgtcagttcc

SEQ ID NO: 52 - protein, 117 aa, synthetic construct
QIQLVQSGPELKKPGETVKISCKASGYTFTDYSINWVKRAPGKGLKWMGWINTETREPAYAYDFRGRFAFSLETSASTAYLQINNLKYEDTATYFCALDYSYAMDYWGQGTSVTVSS

SEQ ID NO: 53 - DNA, 1524 bp, synthetic construct
  source 1..1524: mol_type = other DNA
atgcttctcctggtgacaagccttctgctctgtgagttaccacacccagcattcctcctgatcccaattgtgctcactcagtcacctcccagcctggccatgagcctgggaaaaagggccaccatctcctgtagagccagtgagtccgtcacaatcttggggagccatcttattcactggtatcagcagaagcccgggcagcctccaacccttcttattcagctcgcgtcaaacgtccagacgggtgtacctgccagattttctggtagcgggtcccgcactgattttacactgaccatagatccagtggaagaagacgatgtggccgtgtattattgtctgcagagcagaacgattcctcgcacatttggtgggggtactaagctggagattaagggaagcacgtccggctcagggaagccgggctccggcgagggaagcacgaaggggcaaattcagctggtccagagcggacctgagctgaaaaaacccggcgagactgttaagatcagttgtaaagcatctggctataccttcaccgactacagcataaattgggtgaaacgggcccctggaaagggcctcaaatggatgggttggatcaataccgaaactagggagcctgcttatgcatatgacttccgcgggagattcgccttttcactcgagacatctgcctctactgcttacctccaaataaacaacctcaagtatgaagatacagccacttacttttgcgccctcgactatagttacgccatggactactggggacagggaacctccgttaccgtcagttccgcggccgcattcgtgccggtcttcctgccagcgaagcccaccacgacgccagcgccgcgaccaccaacaccggcgcccaccatcgcgtcgcagcccctgtccctgcgcccagaggcgtgccggccagcggcggggggcgcagtgcacacgagggggctggacttcgcctgtgatatctacatctgggcgcccttggccgggacttgtggggtccttctcctgtcactggttatcaccctttactgcaaccacaggaacaaacggggcagaaagaaactcctgtatatattcaaacaaccatttatgagaccagtacaaactactcaagaggaagatggctgtagctgccgatttccagaagaagaagaaggaggatgtgaactgagagtgaagttcagcaggagcgcagagccccccgcgtaccagcagggccagaaccagctctataacgagctcaatctaggacgaagagaggagtacgatgttttggacaagagacgtggccgggaccctgagatggggggaaagccgagaaggaagaaccctcaggaaggcctgtacaatgaactgcagaaagataagatggcggaggcctacagtgagattgggatgaaaggcgagcgccggaggggcaaggggcacgatggcctttaccagggtctcagtacagccaccaaggacacctacgacgcccttcacatgcaggccctgccccctcgctaa

SEQ ID NO: 54 - protein, 507 aa, synthetic construct
MLLLVTSLLLCELPHPAFLLIPIVLTQSPPSLAMSLGKRATISCRASESVTILGSHLIHWYQQKPGQPPTLLIQLASNVQTGVPARFSGSGSRTDFTLTIDPVEEDDVAVYYCLQSRTIPRTFGGGTKLEIKGSTSGSGKPGSGEGSTKGQIQLVQSGPELKKPGETVKISCKASGYTFTDYSINWVKRAPGKGLKWMGWINTETREPAYAYDFRGRFAFSLETSASTAYLQINNLKYEDTATYFCALDYSYAMDYWGQGTSVTVSSAAAFVPVFLPAKPTTTPAPRPPTPAPTIASQPLSLRPEACRPAAGGAVHTRGLDFACDIYIWAPLAGTCGVLLLSLVITLYCNHRNKRGRKKLLYIFKQPFMRPVQTTQEEDGCSCRFPEEEEGGCELRVKFSRSAEPPAYQQGQNQLYNELNLGRREEYDVLDKRRGRDPEMGGKPRRKNPQEGLYNELQKDKMAEAYSEIGMKGERRRGKGHDGLYQGLSTATKDTYDALHMQALPPR

SEQ ID NO: 55 - DNA, 2799 bp, synthetic construct
  source 1..2799: mol_type = other DNA
atgcttctcctggtgacaagccttctgctctgtgagttaccacacccagcattcctcctgatcccaattgtgctcactcagtcacctcccagcctggccatgagcctgggaaaaagggccaccatctcctgtagagccagtgagtccgtcacaatcttggggagccatcttattcactggtatcagcagaagcccgggcagcctccaacccttcttattcagctcgcgtcaaacgtccagacgggtgtacctgccagattttctggtagcgggtcccgcactgattttacactgaccatagatccagtggaagaagacgatgtggccgtgtattattgtctgcagagcagaacgattcctcgcacatttggtgggggtactaagctggagattaagggaagcacgtccggctcagggaagccgggctccggcgagggaagcacgaaggggcaaattcagctggtccagagcggacctgagctgaaaaaacccggcgagactgttaagatcagttgtaaagcatctggctataccttcaccgactacagcataaattgggtgaaacgggcccctggaaagggcctcaaatggatgggttggatcaataccgaaactagggagcctgcttatgcatatgacttccgcgggagattcgccttttcactcgagacatctgcctctactgcttacctccaaataaacaacctcaagtatgaagatacagccacttacttttgcgccctcgactatagttacgccatggactactggggacagggaacctccgttaccgtcagttccgcggccgcattcgtgccggtcttcctgccagcgaagcccaccacgacgccagcgccgcgaccaccaacaccggcgcccaccatcgcgtcgcagcccctgtccctgcgcccagaggcgtgccggccagcggcggggggcgcagtgcacacgagggggctggacttcgcctgtgatatctacatctgggcgcccttggccgggacttgtggggtccttctcctgtcactggttatcaccctttactgcaaccacaggaacaaacggggcagaaagaaactcctgtatatattcaaacaaccatttatgagaccagtacaaactactcaagaggaagatggctgtagctgccgatttccagaagaagaagaaggaggatgtgaactgagagtgaagttcagcaggagcgcagagccccccgcgtaccagcagggccagaaccagctctataacgagctcaatctaggacgaagagaggagtacgatgttttggacaagagacgtggccgggaccctgagatggggggaaagccgagaaggaagaaccctcaggaaggcctgtacaatgaactgcagaaagataagatggcggaggcctacagtgagattgggatgaaaggcgagcgccggaggggcaaggggcacgatggcctttaccagggtctcagtacagccaccaaggacacctacgacgcccttcacatgcaggccctgccccctcgcggcagtggagagggcagaggaagtctgctaacatgcggtgacgtcgaggagaatcctggcccaatgaccaggctgacagtgctggccctgctggcaggactgctggcaagctccagggccgaggtgcagctggtggagtccggcggcggcctggtgcagcctggagtatccctgaggctgtcttgcgcagcaagcggcttcacctttacatcctacaccatgtcttgggtgagacagaccccaggcaagggactggagtgggtggccttcatcagcggcggaggaggcgacacatactatcctgattccgtgaagggccggtttaccatcagcagagacaactccaagaatacactgtatctgcagatgaactccctgagggcagaggacaccgccgtgtactattgcgccagacacggctacgatggcacatggttcgcctattggggccagggcaccctggtgacagtgtctagcggaggaggaggatctggaggaggaggaagcggaggaggaggatccgacgtgctgacccagagcccatcctctctgtctgccagcgtgggcgatagggtgaccatcacatgtcgcgcctctgagaacatctacagctatctggcctggtaccagcagaagcccggcaagtcccctaagctgctggtgtctaatgcaaagaccctggcagagggagtgccatctaggttctccggctctggcagcggcacccagtttagcctgacaatcagctccctgcagcctgaggatttcgccacatactattgtcagcagcactacgccaccccatatacatttggcggcggcaccaagctggagatcaagaggacagtgggaggaggaggaagcggaggaggaggatccggcggcggcggctctcaaggtcaagatcgccacatgattagaatgcgtcaacttatagatattgttgatcagctgaaaaattatgtgaatgacttggtccctgaatttctgccagctccagaagatgtagagacaaactgtgagtggtcagctttttcctgttttcagaaggcccaactaaagtcagcaaatacaggaaacaatgaaaggataatcaatgtatctattaaaaagctgaagaggaacctctggggcctggcgggcttgaattcctgcccttcatgtgattcttatgagaaaaaaccacccaaagaattcctagaaagattcaaatcacttctccaaaagatgattcatcagcatctgtcctctagaacacacggaagtgaagattcctag

SEQ ID NO: 56 - protein, 932 aa, synthetic construct
MLLLVTSLLLCELPHPAFLLIPIVLTQSPPSLAMSLGKRATISCRASESVTILGSHLIHWYQQKPGQPPTLLIQLASNVQTGVPARFSGSGSRTDFTLTIDPVEEDDVAVYYCLQSRTIPRTFGGGTKLEIKGSTSGSGKPGSGEGSTKGQIQLVQSGPELKKPGETVKISCKASGYTFTDYSINWVKRAPGKGLKWMGWINTETREPAYAYDFRGRFAFSLETSASTAYLQINNLKYEDTATYFCALDYSYAMDYWGQGTSVTVSSAAAFVPVFLPAKPTTTPAPRPPTPAPTIASQPLSLRPEACRPAAGGAVHTRGLDFACDIYIWAPLAGTCGVLLLSLVITLYCNHRNKRGRKKLLYIFKQPFMRPVQTTQEEDGCSCRFPEEEEGGCELRVKFSRSAEPPAYQQGQNQLYNELNLGRREEYDVLDKRRGRDPEMGGKPRRKNPQEGLYNELQKDKMAEAYSEIGMKGERRRGKGHDGLYQGLSTATKDTYDALHMQALPPRGSGEGRGSLLTCGDVEENPGPMTRLTVLALLAGLLASSRAEVQLVESGGGLVQPGVSLRLSCAASGFTFTSYTMSWVRQTPGKGLEWVAFISGGGGDTYYPDSVKGRFTISRDNSKNTLYLQMNSLRAEDTAVYYCARHGYDGTWFAYWGQGTLVTVSSGGGGSGGGGSGGGGSDVLTQSPSSLSASVGDRVTITCRASENIYSYLAWYQQKPGKSPKLLVSNAKTLAEGVPSRFSGSGSGTQFSLTISSLQPEDFATYYCQQHYATPYTFGGGTKLEIKRTVGGGGSGGGGSGGGGSQGQDRHMIRMRQLIDIVDQLKNYVNDLVPEFLPAPEDVETNCEWSAFSCFQKAQLKSANTGNNERIINVSIKKLKRNLWGLAGLNSCPSCDSYEKKPPKEFLERFKSLLQKMIHQHLSSRTHGSEDS

SEQ ID NO: 57 - DNA, 735 bp, synthetic construct
  source 1..735: mol_type = other DNA
gaggttcagctggtggagtctggcggtggcctggtgcagcccgggggctctctccgtttgtcctgtgcagcttctggcttcaacattaaagacacctatatccactgggtgcgtcaggctccgggtaagggcctggagtgggttgcaaggatttatcctacgaatggttatactcgttatgccgatagcgtcaagggccgtttcactataagcgcagacacttcgaaaaacacagcctacctccagatgaacagcctgcgtgctgaggacactgccgtctattattgtagcagatggggtggggacggcttctatgctatggactactggggtcaaggtacactagtcaccgtcagcagcggtggtggtggttctggtggtggtggttctggcggcggcggctccgatatccagatgacccagtccccgagctccctgtccgcctctgtgggcgatagggtcactatcacctgccgtgccagtcaggatgtgaatactgctgtagcctggtatcaacagaaacccggaaaggccccgaaactgctgatttactcggcatccttcctctactctggagtcccttctcgcttctctggttcccgctctgggacggatttcactctgaccatcagctccctgcagccggaagacttcgcaacttattactgtcagcaacactatactactcctccgacgttcggacagggtaccaaggtggagatcaaacgtaccgtg

SEQ ID NO: 58 - protein, 245 aa, synthetic construct
EVQLVESGGGLVQPGGSLRLSCAASGFNIKDTYIHWVRQAPGKGLEWVARIYPTNGYTRYADSVKGRFTISADTSKNTAYLQMNSLRAEDTAVYYCSRWGGDGFYAMDYWGQGTLVTVSSGGGGSGGGGSGGGGSDIQMTQSPSSLSASVGDRVTITCRASQDVNTAVAWYQQKPGKAPKLLIYSASFLYSGVPSRFSGSRSGTDFTLTISSLQPEDFATYYCQQHYTTPPTFGQGTKVEIKRTV

SEQ ID NO: 59 - DNA, 360 bp, synthetic construct
  source 1..360: mol_type = other DNA
gaggttcagctggtggagtctggcggtggcctggtgcagcccgggggctctctccgtttgtcctgtgcagcttctggcttcaacattaaagacacctatatccactgggtgcgtcaggctccgggtaagggcctggagtgggttgcaaggatttatcctacgaatggttatactcgttatgccgatagcgtcaagggccgtttcactataagcgcagacacttcgaaaaacacagcctacctccagatgaacagcctgcgtgctgaggacactgccgtctattattgtagcagatggggtggggacggcttctatgctatggactactggggtcaaggtacactagtcaccgtcagcagc

SEQ ID NO: 60 - protein, 120 aa, synthetic construct [sequence omitted]

SEQ ID NO: 61 - DNA, 45 bp, synthetic construct
  source 1..45: mol_type = other DNA
ggtggtggtggttctggtggtggtggttctggcggcggcggctcc

SEQ ID NO: 62 - protein, 15 aa, synthetic construct
GGGGSGGGGSGGGGS

SEQ ID NO: 63 - DNA, 330 bp, synthetic construct
  source 1..330: mol_type = other DNA
gatatccagatgacccagtccccgagctccctgtccgcctctgtgggcgatagggtcactatcacctgccgtgccagtcaggatgtgaatactgctgtagcctggtatcaacagaaacccggaaaggccccgaaactgctgatttactcggcatccttcctctactctggagtcccttctcgcttctctggttcccgctctgggacggatttcactctgaccatcagctccctgcagccggaagacttcgcaacttattactgtcagcaacactatactactcctccgacgttcggacagggtaccaaggtggagatcaaacgtaccgtg

SEQ ID NO: 64 - protein, 110 aa, synthetic construct
DIQMTQSPSSLSASVGDRVTITCRASQDVNTAVAWYQQKPGKAPKLLIYSASFLYSGVPSRFSGSRSGTDFTLTISSLQPEDFATYYCQQHYTTPPTFGQGTKVEIKRTV

SEQ ID NO: 65 - DNA, 1524 bp, synthetic construct
  source 1..1524: mol_type = other DNA
atgcttctcctggtgacaagccttctgctctgtgagttaccacacccagcattcctcctgatcccagaggttcagctggtggagtctggcggtggcctggtgcagcccgggggctctctccgtttgtcctgtgcagcttctggcttcaacattaaagacacctatatccactgggtgcgtcaggctccgggtaagggcctggagtgggttgcaaggatttatcctacgaatggttatactcgttatgccgatagcgtcaagggccgtttcactataagcgcagacacttcgaaaaacacagcctacctccagatgaacagcctgcgtgctgaggacactgccgtctattattgtagcagatggggtggggacggcttctatgctatggactactggggtcaaggtacactagtcaccgtcagcagcggtggtggtggttctggtggtggtggttctggcggcggcggctccgatatccagatgacccagtccccgagctccctgtccgcctctgtgggcgatagggtcactatcacctgccgtgccagtcaggatgtgaatactgctgtagcctggtatcaacagaaacccggaaaggccccgaaactgctgatttactcggcatccttcctctactctggagtcccttctcgcttctctggttcccgctctgggacggatttcactctgaccatcagctccctgcagccggaagacttcgcaacttattactgtcagcaacactatactactcctccgacgttcggacagggtaccaaggtggagatcaaacgtaccgtggcggccgcattcgtgccggtcttcctgccagcgaagcccaccacgacgccagcgccgcgaccaccaacaccggcgcccaccatcgcgtcgcagcccctgtccctgcgcccagaggcgtgccggccagcggcggggggcgcagtgcacacgagggggctggacttcgcctgtgatatctacatctgggcgcccttggccgggacttgtggggtccttctcctgtcactggttatcaccctttactgcaaccacaggaacaaacggggcagaaagaaactcctgtatatattcaaacaaccatttatgagaccagtacaaactactcaagaggaagatggctgtagctgccgatttccagaagaagaagaaggaggatgtgaactgagagtgaagttcagcaggagcgcagagccccccgcgtaccagcagggccagaaccagctctataacgagctcaatctaggacgaagagaggagtacgatgttttggacaagagacgtggccgggaccctgagatggggggaaagccgagaaggaagaaccctcaggaaggcctgtacaatgaactgcagaaagataagatggcggaggcctacagtgagattgggatgaaaggcgagcgccggaggggcaaggggcacgatggcctttaccagggtctcagtacagccaccaaggacacctacgacgcccttcacatgcaggccctgccccctcgctaa

SEQ ID NO: 66 - protein, 507 aa, synthetic construct
MLLLVTSLLLCELPHPAFLLIPEVQLVESGGGLVQPGGSLRLSCAASGFNIKDTYIHWVRQAPGKGLEWVARIYPTNGYTRYADSVKGRFTISADTSKNTAYLQMNSLRAEDTAVYYCSRWGGDGFYAMDYWGQGTLVTVSSGGGGSGGGGSGGGGSDIQMTQSPSSLSASVGDRVTITCRASQDVNTAVAWYQQKPGKAPKLLIYSASFLYSGVPSRFSGSRSGTDFTLTISSLQPEDFATYYCQQHYTTPPTFGQGTKVEIKRTVAAAFVPVFLPAKPTTTPAPRPPTPAPTIASQPLSLRPEACRPAAGGAVHTRGLDFACDIYIWAPLAGTCGVLLLSLVITLYCNHRNKRGRKKLLYIFKQPFMRPVQTTQEEDGCSCRFPEEEEGGCELRVKFSRSAEPPAYQQGQNQLYNELNLGRREEYDVLDKRRGRDPEMGGKPRRKNPQEGLYNELQKDKMAEAYSEIGMKGERRRGKGHDGLYQGLSTATKDTYDALHMQALPPR

SEQ ID NO: 67 - DNA, 2799 bp, synthetic construct
  source 1..2799: mol_type = other DNA
atgcttctcctggtgacaagccttctgctctgtgagttaccacacccagcattcctcctgatcccagaggttcagctggtggagtctggcggtggcctggtgcagcccgggggctctctccgtttgtcctgtgcagcttctggcttcaacattaaagacacctatatccactgggtgcgtcaggctccgggtaagggcctggagtgggttgcaaggatttatcctacgaatggttatactcgttatgccgatagcgtcaagggccgtttcactataagcgcagacacttcgaaaaacacagcctacctccagatgaacagcctgcgtgctgaggacactgccgtctattattgtagcagatggggtggggacggcttctatgctatggactactggggtcaaggtacactagtcaccgtcagcagcggtggtggtggttctggtggtggtggttctggcggcggcggctccgatatccagatgacccagtccccgagctccctgtccgcctctgtgggcgatagggtcactatcacctgccgtgccagtcaggatgtgaatactgctgtagcctggtatcaacagaaacccggaaaggccccgaaactgctgatttactcggcatccttcctctactctggagtcccttctcgcttctctggttcccgctctgggacggatttcactctgaccatcagctccctgcagccggaagacttcgcaacttattactgtcagcaacactatactactcctccgacgttcggacagggtaccaaggtggagatcaaacgtaccgtggcggccgcattcgtgccggtcttcctgccagcgaagcccaccacgacgccagcgccgcgaccaccaacaccggcgcccaccatcgcgtcgcagcccctgtccctgcgcccagaggcgtgccggccagcggcggggggcgcagtgcacacgagggggctggacttcgcctgtgatatctacatctgggcgcccttggccgggacttgtggggtccttctcctgtcactggttatcaccctttactgcaaccacaggaacaaacggggcagaaagaaactcctgtatatattcaaacaaccatttatgagaccagtacaaactactcaagaggaagatggctgtagctgccgatttccagaagaagaagaaggaggatgtgaactgagagtgaagttcagcaggagcgcagagccccccgcgtaccagcagggccagaaccagctctataacgagctcaatctaggacgaagagaggagtacgatgttttggacaagagacgtggccgggaccctgagatggggggaaagccgagaaggaagaaccctcaggaaggcctgtacaatgaactgcagaaagataagatggcggaggcctacagtgagattgggatgaaaggcgagcgccggaggggcaaggggcacgatggcctttaccagggtctcagtacagccaccaaggacacctacgacgcccttcacatgcaggccctgccccctcgcggcagtggagagggcagaggaagtctgctaacatgcggtgacgtcgaggagaatcctggcccaatgaccaggctgacagtgctggccctgctggcaggactgctggcaagctccagggccgaggtgcagctggtggagtccggcggcggcctggtgcagcctggagtatccctgaggctgtcttgcgcagcaagcggcttcacctttacatcctacaccatgtcttgggtgagacagaccccaggcaagggactggagtgggtggccttcatcagcggcggaggaggcgacacatactatcctgattccgtgaagggccggtttaccatcagcagagacaactccaagaatacactgtatctgcagatgaactccctgagggcagaggacaccgccgtgtactattgcgccagacacggctacgatggcacatggttcgcctattggggccagggcaccctggtgacagtgtctagcggaggaggaggatctggaggaggaggaagcggaggaggaggatccgacgtgctgacccagagcccatcctctctgtctgccagcgtgggcgatagggtgaccatcacatgtcgcgcctctgagaacatctacagctatctggcctggtaccagcagaagcccggcaagtcccctaagctgctggtgtctaatgcaaagaccctggcagagggagtgccatctaggttctccggctctggcagcggcacccagtttagcctgacaatcagctccctgcagcctgaggatttcgccacatactattgtcagcagcactacgccaccccatatacatttggcggcggcaccaagctggagatcaagaggacagtgggaggaggaggaagcggaggaggaggatccggcggcggcggctctcaaggtcaagatcgccacatgattagaatgcgtcaacttatagatattgttgatcagctgaaaaattatgtgaatgacttggtccctgaatttctgccagctccagaagatgtagagacaaactgtgagtggtcagctttttcctgttttcagaaggcccaactaaagtcagcaaatacaggaaacaatgaaaggataatcaatgtatctattaaaaagctgaagaggaacctctggggcctggcgggcttgaattcctgcccttcatgtgattcttatgagaaaaaaccacccaaagaattcctagaaagattcaaatcacttctccaaaagatgattcatcagcatctgtcctctagaacacacggaagtgaagattcctag

SEQ ID NO: 68 - protein, 932 aa, synthetic construct
MLLLVTSLLLCELPHPAFLLIPEVQLVESGGGLVQPGGSLRLSCAASGFNIKDTYIHWVRQAPGKGLEWVARIYPTNGYTRYADSVKGRFTISADTSKNTAYLQMNSLRAEDTAVYYCSRWGGDGFYAMDYWGQGTLVTVSSGGGGSGGGGSGGGGSDIQMTQSPSSLSASVGDRVTITCRASQDVNTAVAWYQQKPGKAPKLLIYSASFLYSGVPSRFSGSRSGTDFTLTISSLQPEDFATYYCQQHYTTPPTFGQGTKVEIKRTVAAAFVPVFLPAKPTTTPAPRPPTPAPTIASQPLSLRPEACRPAAGGAVHTRGLDFACDIYIWAPLAGTCGVLLLSLVITLYCNHRNKRGRKKLLYIFKQPFMRPVQTTQEEDGCSCRFPEEEEGGCELRVKFSRSAEPPAYQQGQNQLYNELNLGRREEYDVLDKRRGRDPEMGGKPRRKNPQEGLYNELQKDKMAEAYSEIGMKGERRRGKGHDGLYQGLSTATKDTYDALHMQALPPRGSGEGRGSLLTCGDVEENPGPMTRLTVLALLAGLLASSRAEVQLVESGGGLVQPGVSLRLSCAASGFTFTSYTMSWVRQTPGKGLEWVAFISGGGGDTYYPDSVKGRFTISRDNSKNTLYLQMNSLRAEDTAVYYCARHGYDGTWFAYWGQGTLVTVSSGGGGSGGGGSGGGGSDVLTQSPSSLSASVGDRVTITCRASENIYSYLAWYQQKPGKSPKLLVSNAKTLAEGVPSRFSGSGSGTQFSLTISSLQPEDFATYYCQQHYATPYTFGGGTKLEIKRTVGGGGSGGGGSGGGGSQGQDRHMIRMRQLIDIVDQLKNYVNDLVPEFLPAPEDVETNCEWSAFSCFQKAQLKSANTGNNERIINVSIKKLKRNLWGLAGLNSCPSCDSYEKKPPKEFLERFKSLLQKMIHQHLSSRTHGSEDS

SEQ ID NO: 69 - protein, 5 aa, synthetic construct
SYTMS

SEQ ID NO: 70 - protein, 17 aa, synthetic construct
FISGGGGDTYYPDSVKG

SEQ ID NO: 71 - protein, 10 aa, synthetic construct
HGYDGTWFAY

SEQ ID NO: 72 - protein, 11 aa, synthetic construct
RASENIYSYLA

SEQ ID NO: 73 - protein, 7 aa, synthetic construct
NAKTLAE

SEQ ID NO: 74 - protein, 9 aa, synthetic construct
QQHYATPYT

SEQ ID NO: 75 - DNA, 21 bp, synthetic construct
  source 1..21: mol_type = other DNA
atgaccaggctgacagtgctg

SEQ ID NO: 76 - DNA, 23 bp, synthetic construct
  source 1..23: mol_type = other DNA
cgctagacactgtcaccagggtg

SEQ ID NO: 77 - DNA, 23 bp, synthetic construct
  source 1..23: mol_type = other DNA
gacgtgctgacccagagcccatc

SEQ ID NO: 78 - DNA, 21 bp, synthetic construct
  source 1..21: mol_type = other DNA
cactgtcctcttgatctccag

SEQ ID NO: 79 - DNA, 43 bp, synthetic construct
  source 1..43: mol_type = other DNA
caaggtcaagatcgccacatgattagggaggaggaggaagcgg

SEQ ID NO: 80 - DNA, 66 bp, synthetic construct
  source 1..66: mol_type = other DNA
ctagtgatggtggtgatgatggtggtgatggtgagagcctccacccccggaatcttcacttccgtg